European Patent Application EP 4 245 315 A1, published September 20, 2023. Title: NOVEL CORONAVIRUS VACCINE BASED ON CONTROLLABLE SECRETORY EXPRESSION OF ATTENUATED SALMONELLA, PREPARATION METHOD THEREFOR, AND APPLICATION THEREOF. Applicant: JIANGSU TARGET BIOMEDICAL RESEARCH INSTITUTE CO., LTD. The sequence listing filed with the application follows.

SEQUENCE LISTING (28 sequences)

SEQ ID NO: 1 - DNA, 385 bp, Artificial Sequence (NirB Promoter)
gagggttaccggcccgatcgttgaacatagcggtccgcaggcggcactgcttacagcaaacggtctgtacgctgtcgtctttgtgatgtgcttcctgttaggtttcgtcagccgtcaccgtcagcataacaccctgacctctcattaattgctcatgccggacggcactatcgtcgtccggccttttcctctcttcccccgctacgtgcatctatttctataaacccgctcattttgtctattttttgcacaaacatgaaatatcagacaattccgtgacttaagaaaatttatacaaatcagcaatatacccattaaggagtatataaaggtgaatttgatttacatcaataagcggggttgctgaatcgttaaggtaggcggt

SEQ ID NO: 2 - DNA, 397 bp, Artificial Sequence (SseA Promoter)
agaagagaacaacggcaagttacaggatccgcagcaatatcagcaaaacaccttattgcttgaagcgatcgagcaggccgaaaatatcatcaacattatttattatcgttaccataacagcgcacttgtagtgagtgagcaagagtaaagtaaaaatatcttagagcctatcccaccaggcgttaattggcgcagccagtttggacacggatagcgcgcaaaaaccgcagcgtacacgtagtacgtgaggtttgactcgctacgctcgcccttcgggccgccgctagcggcgttcaaaacgctaacgcgttttggcgagcactgcccaggttcaaaatggcaagtaaaatagccctaatgggataggctcttagttagcacgttaattatctatcgt

SEQ ID NO: 3 - DNA, 374 bp, Artificial Sequence (SseJ Promoter)
tcacataaaacactagcactttagcaataatagtcggatgataagtttgtctgtttttcctgagtatcaagccagctcatactcacgccagcacactaaaatcaggagtggcttcttttttagatctttgccttagccaggcgcacactcaataatgatagcagtcagataatatgtaccaggcattaacctcacgttgttgatgatatatttacttcgttgaaaaacaataaacattgtatgtattttattggcgacgaaaaactgttaaagaagcgtaattccatatacaccatttacctgattacttttcttgctaatatttgctaattaattatttgctaaagcgtgtttaataaagtaaggaggacact

SEQ ID NO: 4 - DNA, 388 bp, Artificial Sequence (SifB Promoter)
ctgccctaccgctaaacatctcattgttgttagcctaataatacttttagtttaacttcttataagacaatttctacacggttgagcaactatttactttctctaaaaataatatagtgcgtaattaatcattactcatagtacatgatgatgtgagaattaagaaaaccgttttactttcattcgttttatctgacatatttcatggccaggaggcgtgggcatgactaaagctacgggtcgatttgaacaattgaacaataatgttgacggttcaggacaaagcaaaaatcaggtgtttcaccgataggcaaaccgatgggcaacatgggataatatttcgaataccacctattccagtaatgaagtatcatataatcacttgtgg

SEQ ID NO: 5 - DNA, 1224 bp, Artificial Sequence (SseJ Signal Peptide)
atgccattgagtgttggacagggttatttcacatcatctatcagttctgaaaaatttaatgcgataaaagaaagcgcacgccttccggaattaagtttatgggagaaaatcaaagcatatttctttaccacccaccatgcagaggcgctcgaatgtatctttaatctttaccaccatcaggaactgaatctaacaccggtacaggttcgcggagcctacatcaaacttcgagccttagcgtctcagggatgtaaagaacagtttattatagaatcacaggaacacgccgataagttgattattaaagatgataatggtgaaaatattttgtctattgaggttgaatgtcatccggaagcttttggtcttgcaaaagaaatcaataaatcacatcccaagcccaaaaatatttctttgggtgatattaccagactggtattttttggcgacagcttgtctgactccttagggcgtatgtttgaaaaaacacatcatatcttaccctcctatggtcaatactttggcggaaggtttactaatggatttacctggactgagtttttatcatctccacacttcttaggtaaagagatgcttaattttgctgaagggggaagtacatcggcaagctattcctgctttaattgcatcggtgactttgtatcaaatacggacagacaagtcgcatcttacaccccttctcaccaggacctggcgatatttttattgggggctaatgactatatgacactacacaaagataatgtaataatggtcgttgagcaacaaattgatgatattgaaaaaataatttccggtggagttaataatgttctggtcatggggattcccgatttgtctttaacaccttatggcaaacattctgatgaaaaaagaaagcttaaggatgaaagcatcgctcacaatgccctgttaaaaactaatgttgaagaattaaaagaaaaatacccccagcataaaatatgctattacgagactgccgatgcatttaaggtgataatggaggcggccagtaatattggttatgatacggaaaacccttatactcaccacggctatgtacatgttcccggggctaaagaccctcagctagatatatgtccgcaatacgtcttcaacgaccttgtccatccaacccaggaagtccatcattgttttgccataatgttagaaagttttatagctcatcattattccactgaa

SEQ ID NO: 6 - DNA, 576 bp, Artificial Sequence (RBD)
ccgaacatcaccaacctgtgcccgtttggcgaggttttcaacgcgacccgtttcgcgagcgtgtatgcgtggaaccgtaaacgtatcagcaactgcgttgcggactatagcgtgctgtacaacagcgcgagcttcagcacctttaagtgctatggtgtgagcccgaccaaactgaacgatctgtgctttaccaacgtttacgcggatagcttcgtgattcgtggcgacgaggttcgtcagatcgcgccgggtcaaaccggcaagattgcggactacaactataaactgccggacgatttcaccggctgcgttatcgcgtggaacagcaacaacctggatagcaaagtgggtggcaactacaactatctgtaccgtctgtttcgtaagagcaacctgaaaccgttcgagcgtgacattagcaccgaaatctaccaggcgggtagcaccccgtgcaacggtgttgagggctttaactgctatttcccgctgcaaagctacggtttccaaccgaccaacggtgttggttaccagccgtaccgtgtggttgtgctgagctttgaactgctgcacgcgccg

SEQ ID NO: 7 - DNA, 870 bp, Artificial Sequence (NTD)
gtgaatctgaccacccgcacccaactgccgccggcgtacaccaacagcttcacccgtggtgtttactatccggacaaagtttttcgtagcagcgtgctgcacagcacccaggacctgttcctgccgttctttagcaacgttacctggttccacgcgatccacgtgagcggcaccaacggcaccaagcgtttcgacaacccggtgctgccgtttaacgatggtgtttacttcgcgagcaccgagaagagcaacatcattcgtggttggatttttggcaccaccctggacagcaaaacccagagcctgctgatcgttaacaacgcgaccaacgtggttattaaggtgtgcgagttccaattttgcaacgatccgttcctgggcgtttactatcacaagaacaacaaaagctggatggagagcgaatttcgtgtttatagcagcgcgaacaactgcacctttgagtacgtgagccagccgttcctgatggacctggaaggcaagcaaggcaacttcaaaaacctgcgtgagttcgtgttcaagaacattgatggttacttcaaaatctacagcaagcacaccccgatcaacctggttcgtgacctgccgcagggttttagcgcgctggagccgctggttgacctgccgatcggtattaacatcacccgttttcaaaccctgctggcgctgcaccgtagctacctgacgccgggtgacagcagcagcggttggaccgctggtgctgcggcgtactatgttggttacctgcaaccgcgtaccttcctgctgaaatacaacgaaaacggcaccatcaccgatgcggttgattgcgcgctggacccgctgagcgaaaccaagtgcaccctgaagagc

SEQ ID NO: 8 - DNA, 576 bp, Artificial Sequence (S2)
ggtgcgggtgcggcgctgcaaatcccgtttgcgatgcaaatggcgtatcgtttcaacggtattggcgttacccagaacgtgctgtacgagaaccagaagctgatcgcgaaccaatttaacagcgcgattggtaaaatccaggatagcctgagcagcaccgcgagcgcgctgggcaaactgcaagatgttgtgaaccagaacgcgcaagcgctgaacaccctggttaagcagctgagcagcaacttcggtgcgattagcagcgtgctgaacgacatcctgagccgtctggacaaagttgaggcggaagtgcaaattgaccgtctgatcaccggccgtctgcaaagcctgcaaacctatgtgacccagcaactgattcgtgcggcggaaattcgtgcgagcgcgaacctggcggcgaccaagatgagcgagtgcgttctgggtcagagcaagcgtgtggacttttgcggtaaaggctatcacctgatgagcttcccgcagagcgcgccgcacggcgttgtgtttctgcacgttacctacgtgccggcgcaagaaaagaactttaccaccgcgccggcg

SEQ ID NO: 9 - DNA, 45 bp, Artificial Sequence (Linker)
ggcggagggggtagcggtggtggcggcagcggaggtggaggcagc

SEQ ID NO: 10 - DNA, 1997 bp, Artificial Sequence (AT)
gcccgggggatccgatactctctcctttcatcgaaataaccctatgaaaaatatggctgcaatcatcttgaatagtagactcacaagggctaatacaaagcgccaaaagaccaaacaaaataccagtattgccaaaaatactacgaagtttaaatgcacagctgcagcatggcgcataagtatttcgccaacaaataggactgacaatagaggaatgattttattcatatggatctccttctttctcttaggttatcgggtgttgcccgcttatttcgcaccacctaagcggcgggggcggttggagcgattggtgcgaaataagaaccattcccttagttactaggttttttgtccttatttcacacattctcacttttcggtataaatgattattgccttttttcctctcaaatcgttgatatggcattcgtttacggtcaagttcaggatccataagcgactaatgccaattgcaataggaaataaacggttacccgttacgttggatgaaaagagacaaaaagaattgcagcaactaaagcagaagtacggcaaaagtgaatccaggattatgtgtattgcgttagatttattgattgcccaagaaaaagcaggatttgaggtaccagcactcaaaaagtgacgtcaccttttatcctaaaaactaaaagtgatagcacttttaattataagaagttagaatattaatcatttgcttaattgtacaatataatgtacaattgttttatagaaataaataaggggtgaaaggaatggaagcagtagcttattcaaatttccgccaaaatttacgtagttatatgaaacaagttaatgaggatgctgaaacacttattgtaacaagtaaagatgtagaagatacagttgttgtattatcaaaaagagattatgattctatgcaagaaacgttgagaacactttctaataattacgtcatggaaaaaattcgtcgaggagatgaacaattctccaaaggtgcatttaaaacacatgacttaatcgaggttgaatctgatgattaaggcttggtctgatgatgcttgggatgattatctttattggcatgagcaaggaaacaaaagcaatataaaaaagattaacaagttaataaaagatatcgatcgttccccctttgctggattaggaaaacctgagccattaaagcatgatttatctggaaaatggtccagaagaattacagatgaacatagactgatatatagagttgaaaatgaaacgatatttatttattctgcaaaagatcactattaaccaatcggaagtaaggaaagggtcagaaacttaaaagtttttgatccttattttatttaccctagtcatttaaaaagctaatatagcttagtgttgattgttattaatgaatgtgtttgttacgcgtattacggatataaggttagtaaaatcatttctaaagttgaggaaaagtaaatataaatggcttaaatttcaacaatttgaagttgaatagatatgttataatactattgtagtgtgggatgttagttactaaaggatgacgcttatatatatgactgaatagaataagcaataggtttaataatctattttaaattttttgtactagttttagtcaattagcaaaaacaacaaaaataaacttctcatagaatttagctaaaaattaatgatttatttacatattaaatttggatacagttaagtaatttttatatattggaggagaagtaatggaatataaatttaacttgaatttgaaagaagtatcgagctcggaagcttggcagcggccgctggcgggtgtgtcgagtggatggtaggatcgacaaagatctggctacactcgatcagcagttagataataaaatcgctatccatcgaagatggatgtgtgttggttttttgtgtgtgtaacgcaacgattgatagcataaccccttggggcctctaaacgggtcttgaggggttttttg

SEQ ID NO: 11 - DNA, 40 bp, Artificial Sequence (PNirB P1 Primer)
gcaaaatcccttataagaattgagggttaccggcccgatc

SEQ ID NO: 12 - DNA, 40 bp, Artificial Sequence (PNirB P2 Primer)
cctctttctctagtatctagaccgcctaccttaacgattc

SEQ ID NO: 13 - DNA, 40 bp, Artificial Sequence (PSseA P1)
caaaatcccttataagaattagaagagaacaacggcaagt

SEQ ID NO: 14 - DNA, 40 bp, Artificial Sequence (PSseA P2 Primer)
tgtccaacactcaatggcatacgatagataattaacgtgc

SEQ ID NO: 15 - DNA, 40 bp, Artificial Sequence (PsifB P1 Primer)
caaaatcccttataagaattctgccctaccgctaaacatc

SEQ ID NO: 16 - DNA, 40 bp, Artificial Sequence (PsifB P2 Primer)
tgtccaacactcaatggcatccacaagtgattatatgata

SEQ ID NO: 17 - DNA, 40 bp, Artificial Sequence (sseJ P1 Primer)
tatcatataatcacttgtggatgccattgagtgttggaca

SEQ ID NO: 18 - DNA, 40 bp, Artificial Sequence (sseJ P2)
gccttcagtggaataatgatgagctataaaactttctaac

SEQ ID NO: 19 - DNA, 40 bp, Artificial Sequence (PsseJ-sseJ P1 Primer)
caaaatcccttataagaatttcacataaaacactagcact

SEQ ID NO: 20 - DNA, 40 bp, Artificial Sequence (PsseJ-sseJ P2 Primer); identical to SEQ ID NO: 18

SEQ ID NO: 21 - DNA, 36 bp, Artificial Sequence (RBD P1 Primer)
agcggaggtggaggcagcccgaacatcaccaacctg

SEQ ID NO: 22 - DNA, 38 bp, Artificial Sequence (RBD P2 Primer)
tctggaacatcgtatgggtacggcgcgtgcagcagttc

SEQ ID NO: 23 - DNA, 38 bp, Artificial Sequence (NTD P1 Primer)
gcagcggaggtggaggcagcgtgaatctgaccacccgc

SEQ ID NO: 24 - DNA, 39 bp, Artificial Sequence (NTD P2 Primer)
tctggaacatcgtatgggtagctcttcagggtgcacttg

SEQ ID NO: 25 - DNA, 36 bp, Artificial Sequence (S2 P1 Primer)
agcggaggtggaggcagcggtgcgggtgcggcgctg

SEQ ID NO: 26 - DNA, 40 bp, Artificial Sequence (S2 P2 Primer)
tctggaacatcgtatgggtacgccggcgcggtggtaaagt

SEQ ID NO: 27 - DNA, 25 bp, Artificial Sequence (Vec P1 Primer)
tacccatacgatgttccagattacg

SEQ ID NO: 28 - DNA, 20 bp, Artificial Sequence (Vec P2 Primer)
gctgcctccacctccgctgc